European Patent Specification EP 3 681 897 B1, published May 14, 2025. Title: N4-modifikuoti citidino nukleotidai ir jø panaudojimas. Applicant: Vilniaus Universitetas. The sequence listing filed with the application follows.

SEQUENCE LISTING (9 sequences)

SEQ ID NO: 1 - protein, 631 aa, Unknown
  Metagenomic origin
MSSLFIGQVFAKTPEVQTSDLTGNTTCSNLVGMVIPADEIGLPTSGATITSATLKIVEDGAIKDAEYCEVLGAIHPVDPTAPDINFQVNLPTNWNKKFLQFGGGYFNGTVRTGLGNPPAGDRKLGKNTPLAQGYVTFGSDSGNSTAPLDASFGMNDEALKNFAGDQLKKTKDVALALANVRYNAVPDQVYFAGGSEGGREGLFIVQNFPDEYDGVISVYPVLNWIPKALKDNRDAQALYKNDGEGWISPEENDLINETVFKACDSLDGVKDGIISNTSECAEKEDKILDTLSESLSEKQIEVIKSFNGPMEFDIQLANDFTTMPGYSQLQGADIGRLFGTRPIPGVPPVVSESVGHVIDEQDALMGVYSDQVIRYKITRNPDFNTLTFDPNEYREEILKASNLLDVTDPNISEFRENGGKLILVHGTEDEMVAPQGTSDYYSKLVNEFGQESLDEFAQYYLVPGFSHGGGNFTMSANLLGALDAWVVNGDVPSNLVAEDQNSATFGRTRPLCEYPTYPQYNGSGDVNSAASFTCLKADKDKDISASDIQKLIEKFEVDGEFANHGTARSLQAHLDILIKLESQERETVDQIVKHTQKFIKLLDNHKKNGKITDHAYNTLKELAESYIKQIK

SEQ ID NO: 2 - protein, 127 aa, Unknown
  Metagenomic origin
MEQLKFQKNWNNKCSCDFFTTIRLKGPKYTVGKELEMRIYKGGVFQNHGMIRVASLRPIQLHQINEWISRLDSGLSPEELRSELFYMYKDKVADVNKVDFYLILCERVKSKPIQNALFSTESTPAHD

SEQ ID NO: 3 - protein, 103 aa, Escherichia coli
MQPNDITFFQRFQDDILAGRKTITIRDESESHFKTGDVLRVGRFEDDGYFCTIEVTATSTVTLDTLTEKHAEQENMTLTELKKVIADIYPGQTQFYVIEFKCL

SEQ ID NO: 4 - DNA, 35 bp, Artificial Sequence
  Template A
ccggaattaaaatctccctatagtgagtcgtatta

SEQ ID NO: 5 - DNA, 35 bp, Artificial Sequence
  Template G
ccggaattggggtctccctatagtgagtcgtatta

SEQ ID NO: 6 - DNA, 35 bp, Artificial Sequence
  Template C
ccggaattcccctctccctatagtgagtcgtatta

SEQ ID NO: 7 - DNA, 35 bp, Artificial Sequence
  Template T
ccggaatttttttctccctatagtgagtcgtatta

SEQ ID NO: 8 - DNA, 23 bp, Artificial Sequence
  T7 promoter primer
taatacgactcactatagggaga

SEQ ID NO: 9 - DNA, 20 bp, Artificial Sequence
  T7 terminator primer
ctagttattgctcagcggtg